European Patent Application EP 4 736 886 A1, published May 6, 2026. Title: 制备抗体偶联小分子药物的方法及其应用. Applicant: 上海偌妥生物科技有限公司. Application CN. The sequence listing filed with the application follows.

SEQUENCE LISTING (36 sequences)

SEQ ID NO: 1 - protein, 227 aa, Homo sapiens
DKTHTCPPCPAPELLGGPSVFLFPPKPKDTLMISRTPEVTCVVVDVSHEDPEVKFNWYVDGVEVHNAKTKPREEQYNSTYRVVSVLTVLHQDWLNGKEYKCKVSNKALPAPIEKTISKAKGQPREPQVYTLPPSREEMTKNQVSLTCLVKGFYPSDIAVEWESNGQPENNYKTTPPVLDSDGSFFLYSKLTVDKSRWQQGNVFSCSVMHEALHNHYTQKSLSLSPGK

SEQ ID NO: 2 - protein, 137 aa, synthetic construct
MGWSLILLFLVAVATRVHSQVQLVESGGGLVQPGGSLRLSCAASGITFPVNAYGWYRQAPGKQRDLVAIISAGGTTNYADSVKGRFTISRDNSKNTLYLQMNSLRAEDTAVYYCYLQRRIGMLRDYWGQGTQVTVSS

SEQ ID NO: 3 - protein, 136 aa, synthetic construct
MGWSLILLFLVAVATRVHSEVQLVESGGGLVKPGGSLRLSCAASGSTSSINAMAWYRQAPGKQREFVAGVTSSGSIVRENYAFYVKGRFTISRDNAKNSLYLQMNSLRAEDTAVYYCNAIPPYSTWGQGTQVTVSS

SEQ ID NO: 4 - protein, 228 aa, Homo sapiens
ERKCCVECPPCPAPPVAGPSVFLFPPKPKDTLMISRTPEVTCVVVDVSHEDPEVQFNWYVDGVEVHNAKTKPREEQFNSTFRVVSVLTVVHQDWLNGKEYKCKVSNKGLPAPIEKTISKTKGQPREPQVYTLPPSREEMTKNQVSLTCLVKGFYPSDIAVEWESNGQPENNYKTTPPMLDSDGSFFLYSKLTVDKSRWQQGNVFSCSVMHEALHNHYTQKSLSLSPGK

SEQ ID NO: 5 - protein, 229 aa, Homo sapiens
ESKYGPPCPSCPAPEFLGGPSVFLFPPKPKDTLMISRTPEVTCVVVDVSQEDPEVQFNWYVDGVEVHNAKTKPREEQFNSTYRVVSVLTVLHQDWLNGKEYKCKVSNKGLPSSIEKTISKAKGQPREPQVYTLPPSQEEMTKNQVSLTCLVKGFYPSDIAVEWESNGQPENNYKTTPPVLDSDGSFFLYSRLTVDKSRWQEGNVFSCSVMHEALHNHYTQKSLSLSLGK

SEQ ID NO: 6 - protein, 12 aa, synthetic construct
ERKCCVECPPCP

SEQ ID NO: 7 - protein, 12 aa, synthetic construct
ERKSCVECPPCP

SEQ ID NO: 8 - protein, 12 aa, synthetic construct
ERKCSVECPPCP

SEQ ID NO: 9 - protein, 12 aa, synthetic construct
ERKCCVESPPCP

SEQ ID NO: 10 - protein, 12 aa, synthetic construct
ERKCCVECPPSP

SEQ ID NO: 11 - protein, 13 aa, synthetic construct
ERKCACVECPPCP

SEQ ID NO: 12 - protein, 14 aa, synthetic construct
ERKCAACVECPPCP

SEQ ID NO: 13 - protein, 15 aa, synthetic construct
ERKCAAACVECPPCP

SEQ ID NO: 14 - protein, 16 aa, synthetic construct
ERKCAAAACVECPPCP

SEQ ID NO: 15 - protein, 17 aa, synthetic construct
ERKCAAAAACVECPPCP

SEQ ID NO: 16 - protein, 18 aa, synthetic construct
ERKCAAAAAACVECPPCP

SEQ ID NO: 17 - protein, 19 aa, synthetic construct
ERKCAAAAAAACVECPPCP

SEQ ID NO: 18 - protein, 20 aa, synthetic construct
ERKCAAAAAAAACVECPPCP

SEQ ID NO: 19 - protein, 21 aa, synthetic construct
ERKCAAAAAAAAACVECPPCP

SEQ ID NO: 20 - protein, 22 aa, synthetic construct
ERKCAAAAAAAAAACVECPPCP

SEQ ID NO: 21 - protein, 23 aa, synthetic construct
ERKCAAAAAAAAAAACVECPPCP

SEQ ID NO: 22 - protein, 24 aa, synthetic construct
ERKCAAAAAAAAAAAACVECPPCP

SEQ ID NO: 23 - protein, 25 aa, synthetic construct
ERKCAAAAAAAAAAAAACVECPPCP

SEQ ID NO: 24 - protein, 14 aa, synthetic construct
ERKAACCVECPPCP

SEQ ID NO: 25 - protein, 14 aa, synthetic construct
ERKCCAAVECPPCP

SEQ ID NO: 26 - protein, 14 aa, synthetic construct
ERKCSSCVECPPCP

SEQ ID NO: 27 - protein, 14 aa, synthetic construct
ERKCKKCVECPPCP

SEQ ID NO: 28 - protein, 14 aa, synthetic construct
ERKCEECVECPPCP

SEQ ID NO: 29 - protein, 14 aa, synthetic construct
ERKCDDCVECPPCP

SEQ ID NO: 30 - protein, 16 aa, synthetic construct
ERKCEEEECVECPPCP

SEQ ID NO: 31 - protein, 17 aa, synthetic construct
ERKCEEEEECVECPPCP

SEQ ID NO: 32 - protein, 18 aa, synthetic construct
ERKCEEEEEECVECPPCP

SEQ ID NO: 33 - protein, 16 aa, synthetic construct
ERKCDDDDCVECPPCP

SEQ ID NO: 34 - protein, 17 aa, synthetic construct
ERKCDDDDDCVECPPCP

SEQ ID NO: 35 - protein, 18 aa, synthetic construct
ERKCDDDDDDCVECPPCP

SEQ ID NO: 36 - protein, 19 aa, synthetic construct
ERKCDDDDDDDCVECPPCP